European Patent Application EP 4 403 572 A1, published July 24, 2024. Title: 抗人CD3抗体及其应用. Applicant: 江苏先声药业有限公司. The sequence listing filed with the application follows.

SEQUENCE LISTING (143 sequences)

SEQ ID NO: 1 - protein, 119 aa, synthetic construct [sequence omitted]

SEQ ID NO: 2 - protein, 106 aa, synthetic construct [sequence omitted]

SEQ ID NO: 3 - protein, 125 aa, synthetic construct
EVQLVESGGGLVQPGGSLKLSCAASGFTFNKYAMNWVRQAPGKGLEWVARIRSKYNNYATYYADSVKDRFTISRDDSKNTAYLQMNNLKTEDTAVYYCVRHGNFGNSYISYWAYWGQGTLVTVSS

SEQ ID NO: 4 - protein, 109 aa, synthetic construct
QTVVTQEPSLTVSPGGTVTLTCGSSTGAVTSGNYPNWVQQKPGQAPRGLIGGTKFLAPGTPARFSGSLLGGKAALTLSGVQPEDEAEYYCVLWYSNRWVFGGGTKLTVL

SEQ ID NO: 5 - protein, 119 aa, synthetic construct
EVQLVQSGAEVKKPGASVKVSCKASGYTFTNYYIHWVRQAPGQGLEWIGWIYPGDGNTKYNEKFKGRATLTADTSTSTAYLELSSLRSEDTAVYYCARDSYSNYYFDYWGQGTLVTVSS

SEQ ID NO: 6 - protein, 112 aa, synthetic construct
DIVMTQSPDSLAVSLGERATINCKSSQSLLNSRTRKNYLAWYQQKPGQPPKLLIYWASTRESGVPDRFSGSGSGTDFTLTISSLQAEDVAVYYCTQSFILRTFGQGTKVEIK

SEQ ID NO: 7 - protein, 124 aa, synthetic construct
EVQLVESGGGLVQPGRSLRLSCAASGFTFDDYSMHWVRQAPGKGLEWVSGISWNSGSIGYADSVKGRFTISRDNAKNSLYLQMNSLRAEDTALYYCAKYGSGYGKFYYYGMDVWGQGTTVTVSS

SEQ ID NO: 8 - protein, 108 aa, synthetic construct
DIQMTQSPSSLSASVGDRVTITCRASQSISSYLNWYQQKPGKAPKLLIYAASSLQSGVPSRFSGSGSGTDFTLTISSLQPEDFATYYCQQSYSTPPITFGQGTRLEIK

SEQ ID NO: 9 - protein, 123 aa, synthetic construct
EVQLVESGGGLVQPGRSLRLSCAASGFTFDDYAMHWVRQAPGKGLEWVSGISWNSGSIGYADSVKGRFTISRDNAKNSLYLQMNSLRAEDTALYYCAKDSRGYGDYRLGGAYWGQGTLVTVSS

SEQ ID NO: 10 - protein, 107 aa, synthetic construct
EIVMTQSPATLSVSPGERATLSCRASQSVSSNLAWYQQKPGQAPRLLIYGASTRATGIPARFSGSGSGTEFTLTISSLQSEDFAVYYCQQYNNWPWTFGQGTKVEIK

SEQ ID NO: 11 - protein, 125 aa, synthetic construct
EVQLVESGGGLVQPKGSLKLSCAASGFTFNTYAMNWVRQAPGKGLEWVARIRSKYNNYATYYADSVKDRFTISRDDSQSILYLQMNNLKTEDTAMYYCVRHGNFGNSYVSWFAYWGQGTLVTVSS

SEQ ID NO: 12 - protein, 109 aa, synthetic construct
QAVVTQESALTTSPGETVTLTCRSSTGAVTTSNYANWVQEKPDHLFTGLIGGTNKRAPGVPARFSGSLIGDKAALTITGAQTEDEAIYFCALWYSNLWVFGGGTKLTVL

SEQ ID NO: 13 - protein, 330 aa, Homo sapiens
ASTKGPSVFPLAPSSKSTSGGTAALGCLVKDYFPEPVTVSWNSGALTSGVHTFPAVLQSSGLYSLSSVVTVPSSSLGTQTYICNVNHKPSNTKVDKKVEPKSCDKTHTCPPCPAPELLGGPSVFLFPPKPKDTLMISRTPEVTCVVVDVSHEDPEVKFNWYVDGVEVHNAKTKPREEQYNSTYRVVSVLTVLHQDWLNGKEYKCKVSNKALPAPIEKTISKAKGQPREPQVYTLPPSREEMTKNQVSLTCLVKGFYPSDIAVEWESNGQPENNYKTTPPVLDSDGSFFLYSKLTVDKSRWQQGNVFSCSVMHEALHNHYTQKSLSLSPGK

SEQ ID NO: 14 - protein, 107 aa, Homo sapiens [sequence omitted]

SEQ ID NO: 15 - protein, 324 aa, Mus musculus
AKTTPPSVYPLAPGSAAQTNSMVTLGCLVKGYFPEPVTVTWNSGSLSSGVHTFPAVLQSDLYTLSSSVTVPSSTWPSETVTCNVAHPASSTKVDKKIVPRDCGCKPCICTVPEVSSVFIFPPKPKDVLTITLTPKVTCVVVDISKDDPEVQFSWFVDDVEVHTAQTQPREEQFNSTFRSVSELPIMHQDWLNGKEFKCRVNSAAFPAPIEKTISKTKGRPKAPQVYTIPPPKEQMAKDKVSLTCMITDFFPEDITVEWQWNGQPAENYKNTQPIMDTDGSYFVYSKLNVQKSNWEAGNTFTCSVLHEGLHNHHTEKSLSHSPGK

SEQ ID NO: 16 - protein, 107 aa, Mus musculus
RADAAPTVSIFPPSSEQLTSGGASVVCFLNNFYPKDINVKWKIDGSERQNGVLNSWTDQDSKDSTYSMSSTLTLTKDEYERHNSYTCEATHKTSTSPIVKSFNRNEC

SEQ ID NO: 17 - protein, 116 aa, synthetic construct
QIPLVQSGPELKKPGETVKISCKTSGYTFTSYGMSWVKQAPGKGLKWMGWINTYSGVPTYADDFKGRFVFSLDTSASTAFLQINNLKNEDTATYFCARLKNNPFCWGQGSTLTVFS

SEQ ID NO: 18 - protein, 112 aa, synthetic construct
DVLMTQSPLSLPVRLGDQASISCRSSQLILHSNGNTYLEWYLQKPGQSPKLLIYKVSNRFSGVPDRFSGSGSGTDFTLKISRVEAEDLGVYYCFQGSHFPWTFGGGTKLEIK

SEQ ID NO: 19 - protein, 119 aa, synthetic construct
QVQLQQPGTELVKPGASVKLSCKASGYTFTSYWVHWVKQRPGQGLEWIGNINPSDGVTNYNEKFKSRATLTVDKSSSTAYMQLSSLTSEDSAVYYCTRDAYGQYYFDDWGQGTTLTVSS

SEQ ID NO: 20 - protein, 112 aa, synthetic construct
DIVMSQSPSSLVVSAGEKVTMSCKSSQSLLNSRTRKNYLAWYQQKPGQSPKLLIYWASVRDSGVPDRFTGSGSGTDFTLTISNVQAEDLAVYYCIQSYYLRTFGGGTILEIK

SEQ ID NO: 21 - protein, 119 aa, synthetic construct
QVQLQQPGSELVRPGASVKLSCKASGYTFTSYWMHWVKQRPGQGLEWIGNTYPGSGSTNYDEKFKSKATLTVDSSSSTAYMQLSSLTSEDSAVYYCTRDRYGVYYFDYWGQGTTLTVSS

SEQ ID NO: 22 - protein, 112 aa, synthetic construct
DIVMSQSPSSLAVSAGEKVTMSCKSSQSLLNSRTRKNYLAWYQQKPGQSPKLLIYWASTRESGVPDRFSGSGSGTDFTLTISSVQAEDLAVYYCTQSYNLRTFGGGTKLEIK

SEQ ID NO: 23 - protein, 123 aa, synthetic construct
EVKLVESGGGLVQPGASLSLSCAASGFTFTDYYMSWVRQPPGKALEWLAMSRNKAKGHTIEYSSSVKGRFTISRDNSQSILYLQMNALRAEDSATYYCARDTYESYDGYFDVWGAGTTVIVSS

SEQ ID NO: 24 - protein, 112 aa, synthetic construct
DIVMSQSPSSLAVSAGETVTMSCKSSQSLFNSRSRKNYLAWYQQKPGQTPKLLIYWASIRESGVPDRFTGSGSGTDFTLTISSVQAEDLAVYYCKQSYYLYTFGSGTKLEIK

SEQ ID NO: 25 - protein, 122 aa, synthetic construct
EVQLQQSGPELVKPGASVKMSCKASGHTFTSHIMHWVKQKPGQGLEWIGYINPNNDRTEYSEKFKGKATLTSDKSSSTAYMELSSLTSEDSAVYYCAGEAYYSNSLYAMDYWGQGTSVTVSS

SEQ ID NO: 26 - protein, 112 aa, synthetic construct
DIVMSQSPSSLAVSAGEKVTMSCKSSQSLFNSRTRKNYLAWYQQKPGQSPELLIYWASTRESGVPVRFTGSGSGTDFTLTISSVQAEDLAVYYCKQSYYLRTFGGGTKLEVK

SEQ ID NO: 27 - protein, 123 aa, synthetic construct
EVQLVESGGGLVQPKGSLKLSCAASGFTFNTYAMNWVRQAPGKGLEWVGRIRSKINNYATYYGDSVKDRFTISRDDSQSMFYLQMNNLKTEDTAMYYCVIHENYGSISWFAYWGQGTLVTVSA

SEQ ID NO: 28 - protein, 109 aa, synthetic construct
QAVVTQESTLTTSPGETVTLTCRSSTGAVTTSNYANWVQEKPDHLFTGLIGGTNNRAPGVPARFSGSLIGDKAALTITGAQTEDEAIYFCALWYSNHWVFGGGTKLTVL

SEQ ID NO: 29 - protein, 114 aa, synthetic construct
QVQLQQSGAELARPGASVKMSCKASGYIFTMNTMHWVKQRPGQGLEWIGYINPYSGYTKYNQIFKDKATLTADKSSSTAYMRLSSLTSEDSAVYYCLRGGEGVWGQGTTLTVSS

SEQ ID NO: 30 - protein, 112 aa, synthetic construct
DVVMTQTPLTLSVTIGQPASISCKSSQSLLDSDGKTYLNWLLQRPGQSPKRLIYLVSELGSGVPDRFTGSGSGTDFTLKISRVEAEDLGVYYCWQGTHFPRTFGGGTKLEIK

SEQ ID NO: 31 - protein, 5 aa, synthetic construct
SYGMS

SEQ ID NO: 32 - protein, 7 aa, synthetic construct
GYTFTSY

SEQ ID NO: 33 - protein, 8 aa, synthetic construct
GYTFTSYG

SEQ ID NO: 34 - protein, 17 aa, synthetic construct
WINTYSGVPTYADDFKG

SEQ ID NO: 35 - protein, 6 aa, synthetic construct
NTYSGV

SEQ ID NO: 36 - protein, 8 aa, synthetic construct
INTYSGVP

SEQ ID NO: 37 - protein, 7 aa, synthetic construct
LKNNPFC

SEQ ID NO: 38 - protein, 9 aa, synthetic construct
ARLKNNPFC

SEQ ID NO: 39 - protein, 16 aa, synthetic construct
RSSQLILHSNGNTYLE

SEQ ID NO: 40 - protein, 11 aa, synthetic construct
QLILHSNGNTY

SEQ ID NO: 41 - protein, 7 aa, synthetic construct
KVSNRFS

SEQ ID NO: 42 - skipped

SEQ ID NO: 43 - protein, 9 aa, synthetic construct
FQGSHFPWT

SEQ ID NO: 44 - protein, 5 aa, synthetic construct
SYWVH

SEQ ID NO: 45 - protein, 7 aa, synthetic construct
GYTFTSY

SEQ ID NO: 46 - protein, 8 aa, synthetic construct
GYTFTSYW

SEQ ID NO: 47 - protein, 17 aa, synthetic construct
NINPSDGVTNYNEKFKS

SEQ ID NO: 48 - protein, 6 aa, synthetic construct
NPSDGV

SEQ ID NO: 49 - protein, 8 aa, synthetic construct
INPSDGVT

SEQ ID NO: 50 - protein, 10 aa, synthetic construct
DAYGQYYFDD

SEQ ID NO: 51 - protein, 12 aa, synthetic construct
TRDAYGQYYFDD

SEQ ID NO: 52 - protein, 17 aa, synthetic construct
KSSQSLLNSRTRKNYLA

SEQ ID NO: 53 - protein, 12 aa, synthetic construct
QSLLNSRTRKNY

SEQ ID NO: 54 - protein, 7 aa, synthetic construct
WASVRDS

SEQ ID NO: 55 - skipped

SEQ ID NO: 56 - protein, 8 aa, synthetic construct
IQSYYLRT

SEQ ID NO: 57 - protein, 5 aa, synthetic construct
SYWMH

SEQ ID NO: 58 - protein, 7 aa, synthetic construct
GYTFTSY

SEQ ID NO: 59 - protein, 8 aa, synthetic construct
GYTFTSYW

SEQ ID NO: 60 - protein, 17 aa, synthetic construct
NTYPGSGSTNYDEKFKS

SEQ ID NO: 61 - protein, 6 aa, synthetic construct
YPGSGS

SEQ ID NO: 62 - protein, 8 aa, synthetic construct
TYPGSGST

SEQ ID NO: 63 - protein, 10 aa, synthetic construct
DRYGVYYFDY

SEQ ID NO: 64 - protein, 12 aa, synthetic construct
TRDRYGVYYFDY

SEQ ID NO: 65 - protein, 17 aa, synthetic construct
KSSQSLLNSRTRKNYLA

SEQ ID NO: 66 - protein, 12 aa, synthetic construct
QSLLNSRTRKNY

SEQ ID NO: 67 - protein, 7 aa, synthetic construct
WASTRES

SEQ ID NO: 68 - skipped

SEQ ID NO: 69 - protein, 8 aa, synthetic construct
TQSYNLRT

SEQ ID NO: 70 - protein, 5 aa, synthetic construct
DYYMS

SEQ ID NO: 71 - protein, 7 aa, synthetic construct
GFTFTDY

SEQ ID NO: 72 - protein, 8 aa, synthetic construct
GFTFTDYY

SEQ ID NO: 73 - protein, 19 aa, synthetic construct
MSRNKAKGHTIEYSSSVKG

SEQ ID NO: 74 - protein, 8 aa, synthetic construct
RNKAKGHT

SEQ ID NO: 75 - protein, 10 aa, synthetic construct
SRNKAKGHTI

SEQ ID NO: 76 - protein, 12 aa, synthetic construct
DTYESYDGYFDV

SEQ ID NO: 77 - protein, 14 aa, synthetic construct
ARDTYESYDGYFDV

SEQ ID NO: 78 - protein, 17 aa, synthetic construct
KSSQSLFNSRSRKNYLA

SEQ ID NO: 79 - protein, 12 aa, synthetic construct
QSLFNSRSRKNY

SEQ ID NO: 80 - protein, 7 aa, synthetic construct
WASIRES

SEQ ID NO: 81 - skipped

SEQ ID NO: 82 - protein, 8 aa, synthetic construct
KQSYYLYT

SEQ ID NO: 83 - protein, 5 aa, synthetic construct
SHIMH

SEQ ID NO: 84 - protein, 7 aa, synthetic construct
GHTFTSH

SEQ ID NO: 85 - protein, 8 aa, synthetic construct
GHTFTSHI

SEQ ID NO: 86 - protein, 17 aa, synthetic construct
YINPNNDRTEYSEKFKG

SEQ ID NO: 87 - protein, 6 aa, synthetic construct
NPNNDR

SEQ ID NO: 88 - protein, 8 aa, synthetic construct
INPNNDRT

SEQ ID NO: 89 - protein, 13 aa, synthetic construct
EAYYSNSLYAMDY

SEQ ID NO: 90 - protein, 15 aa, synthetic construct
AGEAYYSNSLYAMDY

SEQ ID NO: 91 - protein, 17 aa, synthetic construct
KSSQSLFNSRTRKNYLA

SEQ ID NO: 92 - protein, 12 aa, synthetic construct
QSLFNSRTRKNY

SEQ ID NO: 93 - protein, 7 aa, synthetic construct
WASTRES

SEQ ID NO: 94 - skipped

SEQ ID NO: 95 - protein, 8 aa, synthetic construct
KQSYYLRT

SEQ ID NO: 96 - protein, 5 aa, synthetic construct
TYAMN

SEQ ID NO: 97 - protein, 7 aa, synthetic construct
GFTFNTY

SEQ ID NO: 98 - protein, 8 aa, synthetic construct
GFTFNTYA

SEQ ID NO: 99 - protein, 19 aa, synthetic construct
RIRSKINNYATYYGDSVKD

SEQ ID NO: 100 - protein, 8 aa, synthetic construct
RSKINNYA

SEQ ID NO: 101 - protein, 10 aa, synthetic construct
IRSKINNYAT

SEQ ID NO: 102 - protein, 12 aa, synthetic construct
HENYGSISWFAY

SEQ ID NO: 103 - protein, 14 aa, synthetic construct
VIHENYGSISWFAY

SEQ ID NO: 104 - protein, 14 aa, synthetic construct
RSSTGAVTTSNYAN

SEQ ID NO: 105 - protein, 9 aa, synthetic construct
TGAVTTSNY

SEQ ID NO: 106 - protein, 7 aa, synthetic construct
GTNNRAP

SEQ ID NO: 107 - skipped

SEQ ID NO: 108 - protein, 9 aa, synthetic construct
ALWYSNHWV

SEQ ID NO: 109 - protein, 5 aa, synthetic construct
MNTMH

SEQ ID NO: 110 - protein, 7 aa, synthetic construct
GYIFTMN

SEQ ID NO: 111 - protein, 8 aa, synthetic construct
GYIFTMNT

SEQ ID NO: 112 - protein, 17 aa, synthetic construct
YINPYSGYTKYNQIFKD

SEQ ID NO: 113 - protein, 6 aa, synthetic construct
NPYSGY

SEQ ID NO: 114 - protein, 8 aa, synthetic construct
INPYSGYT

SEQ ID NO: 115 - protein, 5 aa, synthetic construct
GGEGV

SEQ ID NO: 116 - protein, 7 aa, synthetic construct
LRGGEGV

SEQ ID NO: 117 - protein, 16 aa, synthetic construct
KSSQSLLDSDGKTYLN

SEQ ID NO: 118 - protein, 11 aa, synthetic construct
QSLLDSDGKTY

SEQ ID NO: 119 - protein, 7 aa, synthetic construct
LVSELGS

SEQ ID NO: 120 - skipped

SEQ ID NO: 121 - protein, 9 aa, synthetic construct
WQGTHFPRT

SEQ ID NO: 122 - protein, 106 aa, Homo sapiens
GQPKANPTVTLFPPSSEELQANKATLVCLISDFYPGAVTVAWKADGSPVKAGVETTKPSKQSNNKYAASSYLSLTPEQWKSHRSYSCQVTHEGSTVEKTVAPTECS

SEQ ID NO: 123 - protein, 112 aa, synthetic construct
DIVMTQSPDSLAVSLGERATINCKSSQSLFNSRTRKNYLAWYQQKPGQSPKLLIYWASTRESGVPDRFSGSGSGTDFTLTISSLQAEDVAVYYCKQSYYLRTFGGGTKVEIK

SEQ ID NO: 124 - protein, 122 aa, synthetic construct
EVQLVQSGAEVKKPGSSVKVSCKASGHTFSSHIMHWVRQAPGQGLEWMGYINPNNDRTEYSEKFKGRVTITADKSTSTAYMELSSLRSEDTAVYYCAGEAYYSNSLYAMDYWGQGTTVTVSS

SEQ ID NO: 125 - protein, 112 aa, synthetic construct
DIVMTQSPDSLAVSLGERATINCKSSQSLFNSRSRKNYLAWYQQKPGQTPKLLIYWASIRESGVPDRFSGSGSGTDFTLTISSLQAEDVAVYYCKQSYYLYTFGQGTKLEIK

SEQ ID NO: 126 - protein, 123 aa, synthetic construct
EVQLVESGGGVVQPGRSLRLSCAASGFTFTDYYMSWVRQAPGKGLEWVAMSRNKAKGHTIEYSSSVKGRFTISRDNSKNTLYLQMNSLRAEDTAVYYCARDTYESYDGYFDVWGQGTTVTVSS

SEQ ID NO: 127 - protein, 109 aa, synthetic construct
ETVVTQEPSLTVSPGGTVTLTCRSSTGAVTTSNYANWVQQKPGQAFTGLIGGTNNRAPWTPARFSGSLLGGKAALTLSGVQPEDEAEYYCALWYSNHWVFGGGTKLTVL

SEQ ID NO: 128 - protein, 123 aa, synthetic construct
EVQLVESGGGLVQPGGSLKLSCAASGFTFNTYAMNWVRQASGKGLEWVGRIRSKINNYATYYGDSVKDRFTISRDDSKNTFYLQMNSLKTEDTAVYYCVIHENYGSISWFAYWGQGTLVTVSS

SEQ ID NO: 129 - protein, 112 aa, synthetic construct
DVVMTQSPLSLPVTLGQPASISCKSSQSLLDSDGKTYLNWLQQRPGQSPRRLIYLVSELGSGVPDRFSGSGSGTDFTLKISRVEAEDVGVYYCWQGTHFPRTFGGGTKVEIK

SEQ ID NO: 130 - protein, 114 aa, synthetic construct
EVQLVQSGAEVKKPGASVKVSCKASGYTFTMNTMHWVRQAPGQRLEWMGYINPYSGYTKYNQIFKDRVTITADKSASTAYMELSSLRSEDTAVYYCLRGGEGVWGQGTTVTVSS

SEQ ID NO: 131 - protein, 112 aa, synthetic construct
DIVMTQTPLSLPVTPGEPASISCKSSQSLLNSRTRKNYLAWYLQKPGQSPQLLIYWASVRDSGVPDRFSGSGSGTDFTLKISRVEAEDVGVYYCIQSYYLRTFGGGTKVEIK

SEQ ID NO: 132 - protein, 119 aa, synthetic construct
EVQLVQSGAEVKKPGASVKVSCKASGYTFTSYWVHWVRQAPGQRLEWMGNINPSDGVTNYNEKFKSRVTITVDKSASTAYMELSSLRSEDTAVYYCTRDAYGQYYFDNWGQGTTVTVSS

SEQ ID NO: 133 - protein, 112 aa, synthetic construct
DIVMTQSPDSLAVSLGERATINCKSSQSLLNSRTRKNYLAWYQQKPGQSPKLLIYWASTRESGVPDRFSGSGSGTDFTLTISSLQAEDVAVYYCTQSYNLRTFGGGTKVEIK

SEQ ID NO: 134 - protein, 119 aa, synthetic construct
EVQLVQSGAEVKKPGASVKVSCKASGYTFTSYWMHWVRQAPGQGLEWMGNTYPGSGSTNYDEKFKSRVTITVDSSASTAYMELSSLRSEDTAVYYCTRDRYGVYYFDYWGQGTTVTVSS

SEQ ID NO: 135 - protein, 112 aa, synthetic construct
DIVMTQSPDSLAVSLGERATINCRSSQLILHSSGNTYLEWYQQKPGQSPKLLIYKVSNRFSGVPDRFSGSGSGTDFTLTISSLQAEDVAVYYCFQGSHFPWTFGGGTKVEIK

SEQ ID NO: 136 - protein, 116 aa, synthetic construct
EVQLVQSGSELKKPGASVKVSCKTSGYTFTSYGMSWVRQAPGQGLEWMGWINTYSGVPTYAQDFKGRFVFSLDTSVSTAYLQISSLKAEDTAVYYCARLKNNPFVWGQGTTVTVSS

SEQ ID NO: 137 - protein, 17 aa, synthetic construct
WINTYSGVPTYAQDFKG

SEQ ID NO: 138 - protein, 7 aa, synthetic construct
LKNNPFV

SEQ ID NO: 139 - protein, 9 aa, synthetic construct
ARLKNNPFV

SEQ ID NO: 140 - protein, 16 aa, synthetic construct
RSSQLILHSSGNTYLE

SEQ ID NO: 141 - protein, 11 aa, synthetic construct
QLILHSSGNTY

SEQ ID NO: 142 - protein, 10 aa, synthetic construct
DAYGQYYFDN

SEQ ID NO: 143 - protein, 12 aa, synthetic construct
TRDAYGQYYFDN